European Patent Application EP 4 260 866 A1, published October 18, 2023. Title: MACROPHAGE ACTIVATOR. Applicant: SAISEI PHARMA CO., LTD. The sequence listing filed with the application follows.

SEQUENCE LISTING (1 sequence)

SEQ ID NO: 1 - protein, 458 aa, Homo sapiens
LERGRDYEKNKVCKEFSHLGKEDFTSLSLVLYSRKFPSGTFEQVSQLVKEVVSLTEACCAEGADPDCYDTRTSALSAKSCESNSPFPVHPGTAECCTKEGLERKLCMAALKHQPQEFPTYVEPTNDEICEAFRKDPKEYANQFMWEYSTNYGQAPLSLLVSYTKSYLSMVGSCCTSASPTVCFLKERLQLKHLSLLTTLSNRVCSQYAAYGEKKSRLSNLIKLAQKVPTADLEDVLPLAEDITNILSKCCESASEDCMAKELPEHTVKLCDNLSTKNSKFEDCCQEKTAMDVFVCTYFMPAAQLPELPDVELPTNKDVCDPGNTKVMDKYTFELSRRTHLPEVFLSKVLEPTLKSLGECCDVEDSTTCFNAKGPLLKKELSSFIDKGQELCADYSENTFTEYKKKLAERLKAKLPDATPTELAKLVNKHSDFASNCCSINSPPLYCDSEIDAELKNIL